European Patent Specification EP 3 887 519 B1, published November 5, 2025. Title: METHODS OF DETERMINING PH AND CALCIUM OR CHLORIDE CONCENTRATION IN SAMPLES. Applicant: THE UNIVERSITY OF CHICAGO KRISHNAN, Yamuna CHAKRABORTY, Kasturi LEUNG, Ka Ho SAMINATHAN, Anand. The sequence listing filed with the application follows.

SEQUENCE LISTING (24 sequences)

SEQ ID NO: 1 - DNA, 60 bp, Artificial Sequence
  Synthetic oligonucleotide
  misc_feature (1)..(1): 5' Alexa 488
  misc_feature (3)..(3): Bromo cytosine
  misc_feature (9)..(9): Bromo cytosine
  misc_feature (17)..(17): Bromo cytosine
  misc_feature (23)..(23): Bromo cytosine
cccctaacccctaacccctaaccccatatatatcctagaacgacagacaaacagtgagtc

SEQ ID NO: 2 - DNA, 56 bp, Artificial Sequence
  Synthetic oligonucleotide
  misc_feature (1)..(1): 5'  Dibenzocyclooctyne-amine (DBCO)
  misc_feature (30)..(31): iAlexa 647N
gactcactgtttgtctgtcgttctaggataatattttgttatgtgttatgtgttat

SEQ ID NO: 3 - DNA, 32 bp, Artificial Sequence
  Synthetic oligonucleotide
  misc_feature (1)..(1): 5' Alexa 488
ccccaaccccaatacattttacgcctggtgcc

SEQ ID NO: 4 - DNA, 32 bp, Artificial Sequence
  Synthetic oligonucleotide
  misc_feature (32)..(32): 3' Alexa 647
ccgaccgcaggatcctataaaaccccaacccc

SEQ ID NO: 5 - DNA, 38 bp, Artificial Sequence
  Synthetic oligonucleotide
  misc_feature (20)..(21): iDBCON
ttataggatcctgcggtcggggcaccaggcgtaaaatg

SEQ ID NO: 6 - DNA, 57 bp, Artificial Sequence
  Synthetic oligonucleotide
  misc_feature (1)..(1): 5' Oregon Green
ataacacataacacataacaaaatatatatcctagaacgacagacaaacagtgagtc

SEQ ID NO: 7 - DNA, 56 bp, Artificial Sequence; identical to SEQ ID NO: 2
  Synthetic oligonucleotide
  misc_feature (1)..(1): 5' Ca2+ fluorophore
  misc_feature (30)..(31): Second Label

SEQ ID NO: 8 - DNA, 60 bp, Artificial Sequence; identical to SEQ ID NO: 1
  Synthetic oligonucleotide
  misc_feature (1)..(1): 5' First Label

SEQ ID NO: 9 - DNA, 40 bp, Artificial Sequence
  Synthetic oligonucleotide
  misc_feature (20)..(21): Ca2+ fluorophore
ttataggatcctgcggtcggggcaccaggcgtaaaatgta

SEQ ID NO: 10 - DNA, 32 bp, Artificial Sequence; identical to SEQ ID NO: 3
  Synthetic oligonucleotide
  misc_feature (1)..(1): 5' First Label

SEQ ID NO: 11 - DNA, 32 bp, Artificial Sequence; identical to SEQ ID NO: 4
  Synthetic oligonucleotide
  misc_feature (32)..(32): 3' Second Label

SEQ ID NO: 12 - DNA, 57 bp, Artificial Sequence; identical to SEQ ID NO: 6
  Synthetic oligonucleotide
  misc_feature (1)..(1): 5' First Label

SEQ ID NO: 13 - DNA, 7 bp, Artificial Sequence
  Synthetic oligonucleotide
  misc_feature (1)..(1): Greater than or equal to 2 cytosine residues
  misc_feature (2)..(2): A, T, or G
  misc_feature (3)..(3): Greater than or equal to 2 cytosine residues
  misc_feature (4)..(4): A, T, or G
  misc_feature (5)..(5): Greater than or equal to 2 cytosine residues
  misc_feature (6)..(6): A, T, or G
  misc_feature (7)..(7): Greater than or equal to 2 cytosine residues
cncncnc

SEQ ID NO: 14 - DNA, 7 bp, Artificial Sequence
  Synthetic oligonucleotide
  misc_feature (1)..(1): Greater than or equal to 3 cytosine residues
  misc_feature (2)..(2): A, T, or G
  misc_feature (3)..(3): Greater than or equal to 3 cytosine residues
  misc_feature (4)..(4): A, T, or G
  misc_feature (5)..(5): Greater than or equal to 3 cytosine residues
  misc_feature (6)..(6): A, T, or G
  misc_feature (7)..(7): Greater than or equal to 3 cytosine residues
cncncnc

SEQ ID NO: 15 - DNA, 12 bp, Artificial Sequence
  Synthetic oligonucleotide
  misc_feature (1)..(1): 5' BAC-NH2-Lysine
  misc_feature (12)..(12): 3' Lysine-COOH
atcaacactgca

SEQ ID NO: 16 - DNA, 62 bp, Artificial Sequence
  Synthetic oligonucleotide
  misc_feature (29)..(30): iAlexa 647
tattgtgtattgtgtattgttttatatatataggatcttgctgtctggtgtgcagtgttgat

SEQ ID NO: 17 - DNA, 53 bp, Artificial Sequence
  Synthetic oligonucleotide
  misc_feature (53)..(53): 3' Alexa 546
caccagacagcaagatcctatatatataccccaatccccaatccccaatcccc

SEQ ID NO: 18 - DNA, 53 bp, Artificial Sequence; identical to SEQ ID NO: 17
  Synthetic oligonucleotide
  misc_feature (31)..(31): Bromo cytosine
  misc_feature (37)..(37): Bromo cytosine
  misc_feature (45)..(45): Bromo cytosine
  misc_feature (51)..(51): Bromo cytosine

SEQ ID NO: 19 - DNA, 62 bp, Artificial Sequence; identical to SEQ ID NO: 16
  Synthetic oligonucleotide
  misc_feature (29)..(30): iAlexa 647

SEQ ID NO: 20 - DNA, 53 bp, Artificial Sequence; identical to SEQ ID NO: 17
  Synthetic oligonucleotide

SEQ ID NO: 21 - DNA, 38 bp, Artificial Sequence
  Synthetic oligonucleotide
atcaacactgcacaccagacagcaagatcctatatata

SEQ ID NO: 22 - DNA, 12 bp, Artificial Sequence
  Synthetic oligonucleotide
  misc_feature (1)..(1): 5' Cl- fluorophore
  misc_feature (12)..(12): 3' Lysine-COOH
atcaacactgca

SEQ ID NO: 23 - DNA, 62 bp, Artificial Sequence; identical to SEQ ID NO: 16
  Synthetic oligonucleotide
  misc_feature (29)..(30): First Label

SEQ ID NO: 24 - DNA, 53 bp, Artificial Sequence; identical to SEQ ID NO: 17
  Synthetic oligonucleotide
  misc_feature (53)..(53): 3' Second Label